European Patent Specification EP 4 298 240 B1, published June 26, 2024. Title: SPATIAL MAPPING BY SERIAL PRIMER EXTENSION. Applicant: Pixelgen Technologies AB Fredriksson, Simon Karlsson, Filip. The sequence listing filed with the application follows.

SEQUENCE LISTING (27 sequences)

SEQ ID NO: 1 - DNA, 84 bp, Artificial Sequence
  synthetic sequence
  misc_feature (23)..(42): n is a, c, g, or t
gctttaaggccggtcctagcaannnnnnnnnnnnnnnnnnnncaacatcagtattcccaggctacctgcaggttaagcggattg

SEQ ID NO: 2 - DNA, 94 bp, Artificial Sequence
  synthetic sequence
  misc_feature (26)..(45): n is a, c, g, or t
caacatcagtattcccaggctaaaannnnnnnnnnnnnnnnnnnnagatcggaagagcgtcgtgtagggaaagacctgcaggttaagcggattg

SEQ ID NO: 3 - DNA, 42 bp, Artificial Sequence
  synthetic sequence
ttgctaggaccggccttaaagccaatccgcttaacctgcagg

SEQ ID NO: 4 - DNA, 42 bp, Artificial Sequence
  synthetic sequence
tagcctgggaatactgatgttgcaatccgcttaacctgcagg

SEQ ID NO: 5 - DNA, 20 bp, Artificial Sequence
  synthetic sequence
cctgcaggttaagcggattg

SEQ ID NO: 6 - DNA, 52 bp, Artificial Sequence
  synthetic sequence
caagcagaagacggcatacgagatcgagtaatgtgactggagttcagacgtg

SEQ ID NO: 7 - DNA, 61 bp, Artificial Sequence
  synthetic sequence
aatgatacggcgaccaccgagatctacactatagcctacactctttccctacacgacgctc

SEQ ID NO: 8 - DNA, 90 bp, Artificial Sequence
  synthetic sequence
  misc_feature (35)..(44): n is a, c, g, or t
  misc_feature (60)..(68): n is a, c, g, or t
gtgactggagttcagacgtgtgctcttccgatctnnnnnnnnnntcccttgcgatttacnnnnnnnnngctttaaggccggtcctagcaa

SEQ ID NO: 9 - DNA, 90 bp, Artificial Sequence
  synthetic sequence
  misc_feature (35)..(44): n is a, c, g, or t
  misc_feature (60)..(68): n is a, c, g, or t
gtgactggagttcagacgtgtgctcttccgatctnnnnnnnnnntatcccttgggatggnnnnnnnnngctttaaggccggtcctagcaa

SEQ ID NO: 10 - DNA, 90 bp, Artificial Sequence
  synthetic sequence
  misc_feature (35)..(44): n is a, c, g, or t
  misc_feature (60)..(68): n is a, c, g, or t
gtgactggagttcagacgtgtgctcttccgatctnnnnnnnnnnctgggcaattactcgnnnnnnnnngctttaaggccggtcctagcaa

SEQ ID NO: 11 - DNA, 90 bp, Artificial Sequence
  synthetic sequence
  misc_feature (35)..(44): n is a, c, g, or t
  misc_feature (60)..(68): n is a, c, g, or t
gtgactggagttcagacgtgtgctcttccgatctnnnnnnnnnngccggacgacattaannnnnnnnngctttaaggccggtcctagcaa

SEQ ID NO: 12 - DNA, 90 bp, Artificial Sequence
  synthetic sequence
  misc_feature (35)..(44): n is a, c, g, or t
  misc_feature (60)..(68): n is a, c, g, or t
gtgactggagttcagacgtgtgctcttccgatctnnnnnnnnnnttctgggtccctagannnnnnnnngctttaaggccggtcctagcaa

SEQ ID NO: 13 - DNA, 90 bp, Artificial Sequence
  synthetic sequence
  misc_feature (35)..(44): n is a, c, g, or t
  misc_feature (60)..(68): n is a, c, g, or t
gtgactggagttcagacgtgtgctcttccgatctnnnnnnnnnngtctcttggcttaaannnnnnnnngctttaaggccggtcctagcaa

SEQ ID NO: 14 - DNA, 90 bp, Artificial Sequence
  synthetic sequence
  misc_feature (35)..(44): n is a, c, g, or t
  misc_feature (60)..(68): n is a, c, g, or t
gtgactggagttcagacgtgtgctcttccgatctnnnnnnnnnnaatagcgagcaagtannnnnnnnngctttaaggccggtcctagcaa

SEQ ID NO: 15 - DNA, 90 bp, Artificial Sequence
  synthetic sequence
  misc_feature (35)..(44): n is a, c, g, or t
  misc_feature (60)..(68): n is a, c, g, or t
gtgactggagttcagacgtgtgctcttccgatctnnnnnnnnnngctgcgctttccattnnnnnnnnngctttaaggccggtcctagcaa

SEQ ID NO: 16 - DNA, 90 bp, Artificial Sequence
  synthetic sequence
  misc_feature (35)..(44): n is a, c, g, or t
  misc_feature (60)..(68): n is a, c, g, or t
gtgactggagttcagacgtgtgctcttccgatctnnnnnnnnnncaatcagacctatgannnnnnnnngctttaaggccggtcctagcaa

SEQ ID NO: 17 - DNA, 90 bp, Artificial Sequence
  synthetic sequence
  misc_feature (35)..(44): n is a, c, g, or t
  misc_feature (60)..(68): n is a, c, g, or t
gtgactggagttcagacgtgtgctcttccgatctnnnnnnnnnnatatgtatcacgcgannnnnnnnngctttaaggccggtcctagcaa

SEQ ID NO: 18 - DNA, 90 bp, Artificial Sequence
  synthetic sequence
  misc_feature (35)..(44): n is a, c, g, or t
  misc_feature (60)..(68): n is a, c, g, or t
gtgactggagttcagacgtgtgctcttccgatctnnnnnnnnnntcaatccttccgcttnnnnnnnnngctttaaggccggtcctagcaa

SEQ ID NO: 19 - DNA, 90 bp, Artificial Sequence
  synthetic sequence
  misc_feature (35)..(44): n is a, c, g, or t
  misc_feature (60)..(68): n is a, c, g, or t
gtgactggagttcagacgtgtgctcttccgatctnnnnnnnnnnctccgaatcatgttgnnnnnnnnngctttaaggccggtcctagcaa

SEQ ID NO: 20 - DNA, 90 bp, Artificial Sequence
  synthetic sequence
  misc_feature (35)..(44): n is a, c, g, or t
  misc_feature (60)..(68): n is a, c, g, or t
gtgactggagttcagacgtgtgctcttccgatctnnnnnnnnnngtccctgcaacttgannnnnnnnngctttaaggccggtcctagcaa

SEQ ID NO: 21 - DNA, 90 bp, Artificial Sequence
  synthetic sequence
  misc_feature (35)..(44): n is a, c, g, or t
  misc_feature (60)..(68): n is a, c, g, or t
gtgactggagttcagacgtgtgctcttccgatctnnnnnnnnnntcccacttccgctttnnnnnnnnngctttaaggccggtcctagcaa

SEQ ID NO: 22 - DNA, 90 bp, Artificial Sequence
  synthetic sequence
  misc_feature (35)..(44): n is a, c, g, or t
  misc_feature (60)..(68): n is a, c, g, or t
gtgactggagttcagacgtgtgctcttccgatctnnnnnnnnnntggattcccggacttnnnnnnnnngctttaaggccggtcctagcaa

SEQ ID NO: 23 - DNA, 90 bp, Artificial Sequence
  synthetic sequence
  misc_feature (35)..(44): n is a, c, g, or t
  misc_feature (60)..(68): n is a, c, g, or t
gtgactggagttcagacgtgtgctcttccgatctnnnnnnnnnncgcgaacataagaagnnnnnnnnngctttaaggccggtcctagcaa

SEQ ID NO: 24 - DNA, 90 bp, Artificial Sequence
  synthetic sequence
  misc_feature (35)..(44): n is a, c, g, or t
  misc_feature (60)..(68): n is a, c, g, or t
gtgactggagttcagacgtgtgctcttccgatctnnnnnnnnnncagtcgtggtagatannnnnnnnngctttaaggccggtcctagcaa

SEQ ID NO: 25 - DNA, 90 bp, Artificial Sequence
  synthetic sequence
  misc_feature (35)..(44): n is a, c, g, or t
  misc_feature (60)..(68): n is a, c, g, or t
gtgactggagttcagacgtgtgctcttccgatctnnnnnnnnnnatatgtcagagcaccnnnnnnnnngctttaaggccggtcctagcaa

SEQ ID NO: 26 - DNA, 90 bp, Artificial Sequence
  synthetic sequence
  misc_feature (35)..(44): n is a, c, g, or t
  misc_feature (60)..(68): n is a, c, g, or t
gtgactggagttcagacgtgtgctcttccgatctnnnnnnnnnnggtggctagataatgnnnnnnnnngctttaaggccggtcctagcaa

SEQ ID NO: 27 - DNA, 90 bp, Artificial Sequence
  synthetic sequence
  misc_feature (35)..(44): n is a, c, g, or t
  misc_feature (60)..(68): n is a, c, g, or t
gtgactggagttcagacgtgtgctcttccgatctnnnnnnnnnngagatgtctgcaactnnnnnnnnngctttaaggccggtcctagcaa